European Patent Application EP 4 578 876 A1, published July 2, 2025. Title: Bispecific Antibody. Applicant: Ono Pharmaceutical Co., Ltd. Application JP. The sequence listing filed with the application follows.

SEQUENCE LISTING (115 sequences)

SEQ ID NO: 1 - protein, 123 aa, Homo sapiens
EVQLVESGGGLVQPGGSLRLSCAASGIDFSSYYDMCWVRQAPGKCLEWIGCIYTGSVGELYYASWAKGRFTISRDNSKNTVYLQMNSLRAEDTAVYYCARRGSGVDDYYFNLWGQGTLVTVSS

SEQ ID NO: 2 - protein, 121 aa, Homo sapiens
EVQLVESGGGLVQPGGSLRLSCAASGFSLSSHAMAWVRQAPGKGLEWIGYIWSGGITEYPSWAKGRFTISRDNSKNTVYLQMNSLRAEDTAVYYCARDVHIYGDIYAFDLWGQGTLVTVSS

SEQ ID NO: 3 - protein, 119 aa, Homo sapiens
EVQLVESGGGLVQPGGSLRLSCAASGFSLTIYTITWVRQAPGKGLEWIGTINSYGNTYYSTWAKGRFTISRDNSKNTVYLQMNSLRAEDTAVYYCARGYVDSDWYLNIWGQGTLVTVSS

SEQ ID NO: 4 - protein, 119 aa, Homo sapiens; identical to SEQ ID NO: 3

SEQ ID NO: 5 - protein, 119 aa, Homo sapiens
EVQLVESGGGLVQPGGSLRLSCAASGFSLTIYTITWVRQAPGKCLEWIGTINSYGNTYYSTWAKGRFTISRDNSKNTVYLQMNSLRAEDTAVYYCARGYVDSDWYLNIWGQGTLVTVSS

SEQ ID NO: 6 - protein, 119 aa, Homo sapiens
EVQLVESGGGLVQPGGSLRLSCAASGFSLSSYAMIWVRQAPGKGLEWIGFIDTDGHTEYANWAKGRFTISRDNSKNTVYLQMNSLRAEDTAVYYCARDGDHDYWGFNLWGQGTLVTVSS

SEQ ID NO: 7 - protein, 117 aa, Homo sapiens
EVQLVESGGGLVQPGGSLRLSCAASGFSLNNYFMIWVRQAPGKCLEWIGIITSYHTTYFANWAKGRFTISRDNSKNTVYLQMNSLRAEDTAVYYCAPYDIYGYPTLWGQGTLVTVSS

SEQ ID NO: 8 - protein, 119 aa, Homo sapiens
ESQLVESGGGLVQPGGSLRLSCAVSGIDLSSYAVGWVRQAPGKGLEWIGIIGRSGSIYYASWAKGRFTISKDNSKNTVYLQMNSLRAEDTAVYYCARDVDSRPPTGSLWGQGTLVTVSS

SEQ ID NO: 9 - protein, 119 aa, Homo sapiens
EVQLVESGGGLVQPGGSLRLSCAASGIDLSYYAMNWVRQAPGKGLEWIGMIVGGGITFYANWAKGRFTISRDNSKNTVYLQMNSLRAEDTAVYYCAVGSDGGISDFNIWGQGTLVTVSS

SEQ ID NO: 10 - protein, 121 aa, Homo sapiens
EVQLVESGGGLVQPGGSLRLSCAASGFSLSSHAMSWVRQAPGKGLEWIGTISTIDTTYYASWAKGRFTISRDNSKNTVYLQMNSLRAEDTAVYYCARLSELYTTNSYYSRWGQGTLVTVSS

SEQ ID NO: 11 - protein, 121 aa, Homo sapiens
EVQLVESGGGLVQPGGSLRLSCAASGFSLSSHAMSWVRQAPGKCLEWIGTISTIDTTYYASWAKGRFTISRDNSKNTVYLQMNSLRAEDTAVYYCARLSELYTTNSYYSRWGQGTLVTVSS

SEQ ID NO: 12 - protein, 113 aa, Homo sapiens
DIQMTQSPSSLSASVGDRVTITCQSSQSVDNNNWLAWYQQKPGKAPKLLIYDASTLASGVPSRFSGSGSGTDFTLTISSLQPEDFATYYCQGTYYTTDWWNSFGCGTKVTVLG

SEQ ID NO: 13 - protein, 112 aa, Homo sapiens
DIQMTQSPSSLSASVGDRVTITCQASQDIESYLNWYQQKPGKAPKLLIYYASTLASGVPSRFSGSGSGTDFTLTISSLQPEDFATYYCQQSYSNSDVDKNVFGTGTKVTVLG

SEQ ID NO: 14 - protein, 113 aa, Homo sapiens
DIQMTQSPSSLSASVGDRVTITCQSSESVYDNNYLSWYQQKPGKAPKLLIYDASRLASGVPSRFSGSGSGTDFTLTISSLQPEDFATYYCLGGYDSSGWYAAFGTGTKVTVLG

SEQ ID NO: 15 - protein, 113 aa, Homo sapiens
AIQMTQSPSSLSARVGDRVTITCQSSESVYDNNYLSWYQQKPGKAPKLLIYDASRLASGVPSRFSGSGSGTQFTLTISSLQPEDFATYYCLGGYDSSGWYAAFGTGTKVTVLG

SEQ ID NO: 16 - protein, 113 aa, Homo sapiens
AIQMTQSPSSLSARVGDRVTITCQSSESVYDNNYLSWYQQKPGKAPKLLIYDASRLASGVPSRFSGSGSGTQFTLTISSLQPEDFATYYCLGGYDSSGWYAAFGCGTKVTVLG

SEQ ID NO: 17 - protein, 111 aa, Homo sapiens
DIQMTQSPSSLSASVGDRVTITCQASQNIYRNLVWYQQKPGKAPKLLIYGASELESGVPSRFSGSGSGTDFTLTISSLQPEDFATYYCLSTYYISSSDNSFGTGTKVTVLG

SEQ ID NO: 18 - protein, 112 aa, Homo sapiens
DIQMTQSPSSLSASVGDRVTITCQASQSIGAYLSWYQQKPGKAPKLLIYEASTLASGVPSRFSGSGSGTDFTLTISSLQPEDFATYYCLGAYGRSSDDGTAFGCGTKVTVLG

SEQ ID NO: 19 - protein, 111 aa, Homo sapiens
DVQMTQSPSSLSASVGDRVTITCQASQNTYSNLDWYQQKPGKAPKLLIYQASKLASGVPSRFSGSGSGTDFTLTISSLQPEDFATYYCQSTSWGSSYVGGFGTGTKVTVLG

SEQ ID NO: 20 - protein, 111 aa, Homo sapiens
DIQMTQSPSSLSASVGDRVTITCQASQSISSYLAWYQQKPGKAPKLLIYRASTLASGVPSRFSGSGSGTDFTLTISSLQPEDFATYYCQQAYSLSNVDNFFGTGTKVTVLG

SEQ ID NO: 21 - protein, 112 aa, Homo sapiens
DIQMTQSPSSLSASVGDRVTITCQASESIGSLLAWYQQKPGKAPKLLIYRASTLESGVPSRFSGSGSGTDFTLTISSLQPEDFATYYCQSYHYSSSSSYAAFGTGTKVTVLG

SEQ ID NO: 22 - protein, 112 aa, Homo sapiens
DIQMTQSPSSLSASVGDRVTITCQASESIGSLLAWYQQKPGKAPKLLIYRASTLESGVPSRFSGSGSGTDFTLTISSLQPEDFATYYCQSYHYSSSSSYAAFGCGTKVTVLG

SEQ ID NO: 23 - protein, 329 aa, Homo sapiens
ASTKGPSVFPLAPSSKSTSGGTAALGCLVKDYFPEPVTVSWNSGALTSGVHTFPAVLQSSGLYSLSSVVTVPSSSLGTQTYICNVNHKPSNTKVDKRVEPKSCDKTHTCPPCPAPEAAGGPSVFLFPPKPKDTLMISRTPEVTCVVVDVSHEDPEVKFNWYVDGVEVHNAKTKPREEQYASTYRVVSVLTVLHQDWLNGKEYKCKVSNKALPAPIEKTISKAKGQPREPQVYTLPPSREEMTKNQVSLTCLVKGFYPSDIAVEWESNGQPENNYKTTPPVLDSDGSFFLYSKLTVDKSRWQQGNVFSCSVMHEALHNHYTQKSLSLSPG

SEQ ID NO: 24 - protein, 107 aa, Homo sapiens [sequence omitted]

SEQ ID NO: 25 - protein, 11 aa, Homo sapiens
GIDFSSYYDMC

SEQ ID NO: 26 - protein, 18 aa, Homo sapiens
CIYTGSVGELYYASWAKG

SEQ ID NO: 27 - protein, 13 aa, Homo sapiens
RRGSGVDDYYFNL

SEQ ID NO: 28 - protein, 10 aa, Homo sapiens
GFSLSSHAMA

SEQ ID NO: 29 - protein, 16 aa, Homo sapiens
YIWSGGITEYPSWAKG

SEQ ID NO: 30 - protein, 14 aa, Homo sapiens
RDVHIYGDIYAFDL

SEQ ID NO: 31 - protein, 10 aa, Homo sapiens
GFSLTIYTIT

SEQ ID NO: 32 - protein, 16 aa, Homo sapiens
TINSYGNTYYSTWAKG

SEQ ID NO: 33 - protein, 12 aa, Homo sapiens
RGYVDSDWYLNI

SEQ ID NO: 34 - protein, 10 aa, Homo sapiens
GFSLSSYAMI

SEQ ID NO: 35 - protein, 16 aa, Homo sapiens
FIDTDGHTEYANWAKG

SEQ ID NO: 36 - protein, 12 aa, Homo sapiens
RDGDHDYWGFNL

SEQ ID NO: 37 - protein, 10 aa, Homo sapiens
GFSLNNYFMI

SEQ ID NO: 38 - protein, 16 aa, Homo sapiens
IITSYHTTYFANWAKG

SEQ ID NO: 39 - protein, 10 aa, Homo sapiens
PYDIYGYPTL

SEQ ID NO: 40 - protein, 10 aa, Homo sapiens
GIDLSSYAVG

SEQ ID NO: 41 - protein, 16 aa, Homo sapiens
IIGRSGSIYYASWAKG

SEQ ID NO: 42 - protein, 12 aa, Homo sapiens
RDVDSRPPTGSL

SEQ ID NO: 43 - protein, 10 aa, Homo sapiens
GIDLSYYAMN

SEQ ID NO: 44 - protein, 16 aa, Homo sapiens
MIVGGGITFYANWAKG

SEQ ID NO: 45 - protein, 12 aa, Homo sapiens
VGSDGGISDFNI

SEQ ID NO: 46 - protein, 10 aa, Homo sapiens
GFSLSSHAMS

SEQ ID NO: 47 - protein, 16 aa, Homo sapiens
TISTIDTTYYASWAKG

SEQ ID NO: 48 - protein, 14 aa, Homo sapiens
RLSELYTTNSYYSR

SEQ ID NO: 49 - protein, 13 aa, Homo sapiens
QSSQSVDNNNWLA

SEQ ID NO: 50 - protein, 7 aa, Homo sapiens
DASTLAS

SEQ ID NO: 51 - protein, 12 aa, Homo sapiens
QGTYYTTDWWNS

SEQ ID NO: 52 - protein, 11 aa, Homo sapiens
QASQDIESYLN

SEQ ID NO: 53 - protein, 7 aa, Homo sapiens
YASTLAS

SEQ ID NO: 54 - protein, 13 aa, Homo sapiens
QQSYSNSDVDKNV

SEQ ID NO: 55 - protein, 13 aa, Homo sapiens
QSSESVYDNNYLS

SEQ ID NO: 56 - protein, 7 aa, Homo sapiens
DASRLAS

SEQ ID NO: 57 - protein, 12 aa, Homo sapiens
LGGYDSSGWYAA

SEQ ID NO: 58 - protein, 11 aa, Homo sapiens
QASQNIYRNLV

SEQ ID NO: 59 - protein, 7 aa, Homo sapiens
GASELES

SEQ ID NO: 60 - protein, 12 aa, Homo sapiens
LSTYYISSSDNS

SEQ ID NO: 61 - protein, 11 aa, Homo sapiens
QASQSIGAYLS

SEQ ID NO: 62 - protein, 7 aa, Homo sapiens
EASTLAS

SEQ ID NO: 63 - protein, 13 aa, Homo sapiens
LGAYGRSSDDGTA

SEQ ID NO: 64 - protein, 11 aa, Homo sapiens
QASQNTYSNLD

SEQ ID NO: 65 - protein, 7 aa, Homo sapiens
QASKLAS

SEQ ID NO: 66 - protein, 12 aa, Homo sapiens
QSTSWGSSYVGG

SEQ ID NO: 67 - protein, 11 aa, Homo sapiens
QASQSISSYLA

SEQ ID NO: 68 - protein, 7 aa, Homo sapiens
RASTLAS

SEQ ID NO: 69 - protein, 12 aa, Homo sapiens
QQAYSLSNVDNF

SEQ ID NO: 70 - protein, 11 aa, Homo sapiens
QASESIGSLLA

SEQ ID NO: 71 - protein, 7 aa, Homo sapiens
RASTLES

SEQ ID NO: 72 - protein, 13 aa, synthetic construct
QSYHYSSSSSYAA

SEQ ID NO: 73 - protein, 10 aa, synthetic construct
GGGGSGGGGS

SEQ ID NO: 74 - protein, 20 aa, synthetic construct
GGGGSGGGGSGGGGSGGGGS

SEQ ID NO: 75 - protein, 710 aa, Homo sapiens
EVQLVESGGGLVQPGGSLRLSCAASGIDLSYYAMNWVRQAPGKGLEWIGMIVGGGITFYANWAKGRFTISRDNSKNTVYLQMNSLRAEDTAVYYCAVGSDGGISDFNIWGQGTLVTVSSASTKGPSVFPLAPSSKSTSGGTAALGCLVKDYFPEPVTVSWNSGALTSGVHTFPAVLQSSGLYSLSSVVTVPSSSLGTQTYICNVNHKPSNTKVDKRVEPKSCDKTHTCPPCPAPEAAGGPSVFLFPPKPKDTLMISRTPEVTCVVVDVSHEDPEVKFNWYVDGVEVHNAKTKPREEQYASTYRVVSVLTVLHQDWLNGKEYKCKVSNKALPAPIEKTISKAKGQPREPQVYTLPPSREEMTKNQVSLTCLVKGFYPSDIAVEWESNGQPENNYKTTPPVLDSDGSFFLYSKLTVDKSRWQQGNVFSCSVMHEALHNHYTQKSLSLSPGGGGGSGGGGSDIQMTQSPSSLSASVGDRVTITCQSSESVYDNNYLSWYQQKPGKAPKLLIYDASRLASGVPSRFSGSGSGTDFTLTISSLQPEDFATYYCLGGYDSSGWYAAFGTGTKVTVLGGGGGSGGGGSGGGGSGGGGSEVQLVESGGGLVQPGGSLRLSCAASGFSLTIYTITWVRQAPGKGLEWIGTINSYGNTYYSTWAKGRFTISRDNSKNTVYLQMNSLRAEDTAVYYCARGYVDSDWYLNIWGQGTLVTVSS

SEQ ID NO: 76 - protein, 217 aa, Homo sapiens
DIQMTQSPSSLSASVGDRVTITCQASQSISSYLAWYQQKPGKAPKLLIYRASTLASGVPSRFSGSGSGTDFTLTISSLQPEDFATYYCQQAYSLSNVDNFFGQGTKVEIKRTVAAPSVFIFPPSDEQLKSGTASVVCLLNNFYPREAKVQWKVDNALQSGNSQESVTEQDSKDSTYSLSSTLTLSKADYEKHKVYACEVTHQGLSSPVTKSFNRGEC

SEQ ID NO: 77 - protein, 712 aa, Homo sapiens
EVQLVESGGGLVQPGGSLRLSCAASGFSLSSHAMSWVRQAPGKGLEWIGTISTIDTTYYASWAKGRFTISRDNSKNTVYLQMNSLRAEDTAVYYCARLSELYTTNSYYSRWGQGTLVTVSSASTKGPSVFPLAPSSKSTSGGTAALGCLVKDYFPEPVTVSWNSGALTSGVHTFPAVLQSSGLYSLSSVVTVPSSSLGTQTYICNVNHKPSNTKVDKRVEPKSCDKTHTCPPCPAPEAAGGPSVFLFPPKPKDTLMISRTPEVTCVVVDVSHEDPEVKFNWYVDGVEVHNAKTKPREEQYASTYRVVSVLTVLHQDWLNGKEYKCKVSNKALPAPIEKTISKAKGQPREPQVYTLPPSREEMTKNQVSLTCLVKGFYPSDIAVEWESNGQPENNYKTTPPVLDSDGSFFLYSKLTVDKSRWQQGNVFSCSVMHEALHNHYTQKSLSLSPGGGGGSGGGGSDIQMTQSPSSLSASVGDRVTITCQSSESVYDNNYLSWYQQKPGKAPKLLIYDASRLASGVPSRFSGSGSGTDFTLTISSLQPEDFATYYCLGGYDSSGWYAAFGTGTKVTVLGGGGGSGGGGSGGGGSGGGGSEVQLVESGGGLVQPGGSLRLSCAASGFSLTIYTITWVRQAPGKGLEWIGTINSYGNTYYSTWAKGRFTISRDNSKNTVYLQMNSLRAEDTAVYYCARGYVDSDWYLNIWGQGTLVTVSS

SEQ ID NO: 78 - protein, 218 aa, Homo sapiens
DIQMTQSPSSLSASVGDRVTITCQASESIGSLLAWYQQKPGKAPKLLIYRASTLESGVPSRFSGSGSGTDFTLTISSLQPEDFATYYCQSYHYSSSSSYAAFGQGTKVEIKRTVAAPSVFIFPPSDEQLKSGTASVVCLLNNFYPREAKVQWKVDNALQSGNSQESVTEQDSKDSTYSLSSTLTLSKADYEKHKVYACEVTHQGLSSPVTKSFNRGEC

SEQ ID NO: 79 - protein, 712 aa, Homo sapiens
EVQLVESGGGLVQPGGSLRLSCAASGFSLSSHAMSWVRQAPGKGLEWIGTISTIDTTYYASWAKGRFTISRDNSKNTVYLQMNSLRAEDTAVYYCARLSELYTTNSYYSRWGQGTLVTVSSASTKGPSVFPLAPSSKSTSGGTAALGCLVKDYFPEPVTVSWNSGALTSGVHTFPAVLQSSGLYSLSSVVTVPSSSLGTQTYICNVNHKPSNTKVDKRVEPKSCDKTHTCPPCPAPEAAGGPSVFLFPPKPKDTLMISRTPEVTCVVVDVSHEDPEVKFNWYVDGVEVHNAKTKPREEQYASTYRVVSVLTVLHQDWLNGKEYKCKVSNKALPAPIEKTISKAKGQPREPQVYTLPPSREEMTKNQVSLTCLVKGFYPSDIAVEWESNGQPENNYKTTPPVLDSDGSFFLYSKLTVDKSRWQQGNVFSCSVMHEALHNHYTQKSLSLSPGGGGGSGGGGSAIQMTQSPSSLSARVGDRVTITCQSSESVYDNNYLSWYQQKPGKAPKLLIYDASRLASGVPSRFSGSGSGTQFTLTISSLQPEDFATYYCLGGYDSSGWYAAFGCGTKVTVLGGGGGSGGGGSGGGGSGGGGSEVQLVESGGGLVQPGGSLRLSCAASGFSLTIYTITWVRQAPGKCLEWIGTINSYGNTYYSTWAKGRFTISRDNSKNTVYLQMNSLRAEDTAVYYCARGYVDSDWYLNIWGQGTLVTVSS

SEQ ID NO: 80 - protein, 710 aa, Homo sapiens
EVQLVESGGGLVQPGGSLRLSCAASGFSLSSHAMSWVRQAPGKGLEWIGTISTIDTTYYASWAKGRFTISRDNSKNTVYLQMNSLRAEDTAVYYCARLSELYTTNSYYSRWGQGTLVTVSSASTKGPSVFPLAPSSKSTSGGTAALGCLVKDYFPEPVTVSWNSGALTSGVHTFPAVLQSSGLYSLSSVVTVPSSSLGTQTYICNVNHKPSNTKVDKRVEPKSCDKTHTCPPCPAPEAAGGPSVFLFPPKPKDTLMISRTPEVTCVVVDVSHEDPEVKFNWYVDGVEVHNAKTKPREEQYASTYRVVSVLTVLHQDWLNGKEYKCKVSNKALPAPIEKTISKAKGQPREPQVYTLPPSREEMTKNQVSLTCLVKGFYPSDIAVEWESNGQPENNYKTTPPVLDSDGSFFLYSKLTVDKSRWQQGNVFSCSVMHEALHNHYTQKSLSLSPGGGGGSGGGGSDIQMTQSPSSLSASVGDRVTITCQASQNIYRNLVWYQQKPGKAPKLLIYGASELESGVPSRFSGSGSGTDFTLTISSLQPEDFATYYCLSTYYISSSDNSFGTGTKVTVLGGGGGSGGGGSGGGGSGGGGSEVQLVESGGGLVQPGGSLRLSCAASGFSLSSYAMIWVRQAPGKGLEWIGFIDTDGHTEYANWAKGRFTISRDNSKNTVYLQMNSLRAEDTAVYYCARDGDHDYWGFNLWGQGTLVTVSS

SEQ ID NO: 81 - protein, 708 aa, Homo sapiens
EVQLVESGGGLVQPGGSLRLSCAASGFSLTIYTITWVRQAPGKGLEWIGTINSYGNTYYSTWAKGRFTISRDNSKNTVYLQMNSLRAEDTAVYYCARGYVDSDWYLNIWGQGTLVTVSSASTKGPSVFPLAPSSKSTSGGTAALGCLVKDYFPEPVTVSWNSGALTSGVHTFPAVLQSSGLYSLSSVVTVPSSSLGTQTYICNVNHKPSNTKVDKRVEPKSCDKTHTCPPCPAPEAAGGPSVFLFPPKPKDTLMISRTPEVTCVVVDVSHEDPEVKFNWYVDGVEVHNAKTKPREEQYASTYRVVSVLTVLHQDWLNGKEYKCKVSNKALPAPIEKTISKAKGQPREPQVYTLPPSREEMTKNQVSLTCLVKGFYPSDIAVEWESNGQPENNYKTTPPVLDSDGSFFLYSKLTVDKSRWQQGNVFSCSVMHEALHNHYTQKSLSLSPGGGGGSGGGGSDIQMTQSPSSLSASVGDRVTITCQASQSISSYLAWYQQKPGKAPKLLIYRASTLASGVPSRFSGSGSGTDFTLTISSLQPEDFATYYCQQAYSLSNVDNFFGTGTKVTVLGGGGGSGGGGSGGGGSGGGGSEVQLVESGGGLVQPGGSLRLSCAASGIDLSYYAMNWVRQAPGKGLEWIGMIVGGGITFYANWAKGRFTISRDNSKNTVYLQMNSLRAEDTAVYYCAVGSDGGISDFNIWGQGTLVTVSS

SEQ ID NO: 82 - protein, 219 aa, Homo sapiens
DIQMTQSPSSLSASVGDRVTITCQSSESVYDNNYLSWYQQKPGKAPKLLIYDASRLASGVPSRFSGSGSGTDFTLTISSLQPEDFATYYCLGGYDSSGWYAAFGQGTKVEIKRTVAAPSVFIFPPSDEQLKSGTASVVCLLNNFYPREAKVQWKVDNALQSGNSQESVTEQDSKDSTYSLSSTLTLSKADYEKHKVYACEVTHQGLSSPVTKSFNRGEC

SEQ ID NO: 83 - protein, 711 aa, Homo sapiens
EVQLVESGGGLVQPGGSLRLSCAASGFSLTIYTITWVRQAPGKGLEWIGTINSYGNTYYSTWAKGRFTISRDNSKNTVYLQMNSLRAEDTAVYYCARGYVDSDWYLNIWGQGTLVTVSSASTKGPSVFPLAPSSKSTSGGTAALGCLVKDYFPEPVTVSWNSGALTSGVHTFPAVLQSSGLYSLSSVVTVPSSSLGTQTYICNVNHKPSNTKVDKRVEPKSCDKTHTCPPCPAPEAAGGPSVFLFPPKPKDTLMISRTPEVTCVVVDVSHEDPEVKFNWYVDGVEVHNAKTKPREEQYASTYRVVSVLTVLHQDWLNGKEYKCKVSNKALPAPIEKTISKAKGQPREPQVYTLPPSREEMTKNQVSLTCLVKGFYPSDIAVEWESNGQPENNYKTTPPVLDSDGSFFLYSKLTVDKSRWQQGNVFSCSVMHEALHNHYTQKSLSLSPGGGGGSGGGGSDIQMTQSPSSLSASVGDRVTITCQASESIGSLLAWYQQKPGKAPKLLIYRASTLESGVPSRFSGSGSGTDFTLTISSLQPEDFATYYCQSYHYSSSSSYAAFGTGTKVTVLGGGGGSGGGGSGGGGSGGGGSEVQLVESGGGLVQPGGSLRLSCAASGFSLSSHAMSWVRQAPGKGLEWIGTISTIDTTYYASWAKGRFTISRDNSKNTVYLQMNSLRAEDTAVYYCARLSELYTTNSYYSRWGQGTLVTVSS

SEQ ID NO: 84 - protein, 711 aa, Homo sapiens
EVQLVESGGGLVQPGGSLRLSCAASGFSLTIYTITWVRQAPGKGLEWIGTINSYGNTYYSTWAKGRFTISRDNSKNTVYLQMNSLRAEDTAVYYCARGYVDSDWYLNIWGQGTLVTVSSASTKGPSVFPLAPSSKSTSGGTAALGCLVKDYFPEPVTVSWNSGALTSGVHTFPAVLQSSGLYSLSSVVTVPSSSLGTQTYICNVNHKPSNTKVDKRVEPKSCDKTHTCPPCPAPEAAGGPSVFLFPPKPKDTLMISRTPEVTCVVVDVSHEDPEVKFNWYVDGVEVHNAKTKPREEQYASTYRVVSVLTVLHQDWLNGKEYKCKVSNKALPAPIEKTISKAKGQPREPQVYTLPPSREEMTKNQVSLTCLVKGFYPSDIAVEWESNGQPENNYKTTPPVLDSDGSFFLYSKLTVDKSRWQQGNVFSCSVMHEALHNHYTQKSLSLSPGGGGGSGGGGSDIQMTQSPSSLSASVGDRVTITCQASESIGSLLAWYQQKPGKAPKLLIYRASTLESGVPSRFSGSGSGTDFTLTISSLQPEDFATYYCQSYHYSSSSSYAAFGCGTKVTVLGGGGGSGGGGSGGGGSGGGGSEVQLVESGGGLVQPGGSLRLSCAASGFSLSSHAMSWVRQAPGKCLEWIGTISTIDTTYYASWAKGRFTISRDNSKNTVYLQMNSLRAEDTAVYYCARLSELYTTNSYYSRWGQGTLVTVSS

SEQ ID NO: 85 - protein, 219 aa, Homo sapiens
AIQMTQSPSSLSARVGDRVTITCQSSESVYDNNYLSWYQQKPGKAPKLLIYDASRLASGVPSRFSGSGSGTQFTLTISSLQPEDFATYYCLGGYDSSGWYAAFGQGTKVEIKRTVAAPSVFIFPPSDEQLKSGTASVVCLLNNFYPREAKVQWKVDNALQSGNSQESVTEQDSKDSTYSLSSTLTLSKADYEKHKVYACEVTHQGLSSPVTKSFNRGEC

SEQ ID NO: 86 - protein, 711 aa, Homo sapiens
EVQLVESGGGLVQPGGSLRLSCAASGFSLSSYAMIWVRQAPGKGLEWIGFIDTDGHTEYANWAKGRFTISRDNSKNTVYLQMNSLRAEDTAVYYCARDGDHDYWGFNLWGQGTLVTVSSASTKGPSVFPLAPSSKSTSGGTAALGCLVKDYFPEPVTVSWNSGALTSGVHTFPAVLQSSGLYSLSSVVTVPSSSLGTQTYICNVNHKPSNTKVDKRVEPKSCDKTHTCPPCPAPEAAGGPSVFLFPPKPKDTLMISRTPEVTCVVVDVSHEDPEVKFNWYVDGVEVHNAKTKPREEQYASTYRVVSVLTVLHQDWLNGKEYKCKVSNKALPAPIEKTISKAKGQPREPQVYTLPPSREEMTKNQVSLTCLVKGFYPSDIAVEWESNGQPENNYKTTPPVLDSDGSFFLYSKLTVDKSRWQQGNVFSCSVMHEALHNHYTQKSLSLSPGGGGGSGGGGSDIQMTQSPSSLSASVGDRVTITCQASESIGSLLAWYQQKPGKAPKLLIYRASTLESGVPSRFSGSGSGTDFTLTISSLQPEDFATYYCQSYHYSSSSSYAAFGTGTKVTVLGGGGGSGGGGSGGGGSGGGGSEVQLVESGGGLVQPGGSLRLSCAASGFSLSSHAMSWVRQAPGKGLEWIGTISTIDTTYYASWAKGRFTISRDNSKNTVYLQMNSLRAEDTAVYYCARLSELYTTNSYYSRWGQGTLVTVSS

SEQ ID NO: 87 - protein, 217 aa, Homo sapiens
DIQMTQSPSSLSASVGDRVTITCQASQNIYRNLVWYQQKPGKAPKLLIYGASELESGVPSRFSGSGSGTDFTLTISSLQPEDFATYYCLSTYYISSSDNSFGQGTKVEIKRTVAAPSVFIFPPSDEQLKSGTASVVCLLNNFYPREAKVQWKVDNALQSGNSQESVTEQDSKDSTYSLSSTLTLSKADYEKHKVYACEVTHQGLSSPVTKSFNRGEC

SEQ ID NO: 88 - protein, 448 aa, Homo sapiens
EVQLVESGGGLVQPGGSLRLSCAASGIDLSYYAMNWVRQAPGKGLEWIGMIVGGGITFYANWAKGRFTISRDNSKNTVYLQMNSLRAEDTAVYYCAVGSDGGISDFNIWGQGTLVTVSSASTKGPSVFPLAPSSKSTSGGTAALGCLVKDYFPEPVTVSWNSGALTSGVHTFPAVLQSSGLYSLSSVVTVPSSSLGTQTYICNVNHKPSNTKVDKRVEPKSCDKTHTCPPCPAPEAAGGPSVFLFPPKPKDTLMISRTPEVTCVVVDVSHEDPEVKFNWYVDGVEVHNAKTKPREEQYASTYRVVSVLTVLHQDWLNGKEYKCKVSNKALPAPIEKTISKAKGQPREPQVYTLPPSREEMTKNQVSLTCLVKGFYPSDIAVEWESNGQPENNYKTTPPVLDSDGSFFLYSKLTVDKSRWQQGNVFSCSVMHEALHNHYTQKSLSLSPG

SEQ ID NO: 89 - protein, 479 aa, Homo sapiens
DIQMTQSPSSLSASVGDRVTITCQASQSISSYLAWYQQKPGKAPKLLIYRASTLASGVPSRFSGSGSGTDFTLTISSLQPEDFATYYCQQAYSLSNVDNFFGQGTKVEIKRTVAAPSVFIFPPSDEQLKSGTASVVCLLNNFYPREAKVQWKVDNALQSGNSQESVTEQDSKDSTYSLSSTLTLSKADYEKHKVYACEVTHQGLSSPVTKSFNRGECGGGGSGGGGSDIQMTQSPSSLSASVGDRVTITCQSSESVYDNNYLSWYQQKPGKAPKLLIYDASRLASGVPSRFSGSGSGTDFTLTISSLQPEDFATYYCLGGYDSSGWYAAFGTGTKVTVLGGGGGSGGGGSGGGGSGGGGSEVQLVESGGGLVQPGGSLRLSCAASGFSLTIYTITWVRQAPGKGLEWIGTINSYGNTYYSTWAKGRFTISRDNSKNTVYLQMNSLRAEDTAVYYCARGYVDSDWYLNIWGQGTLVTVSS

SEQ ID NO: 90 - protein, 450 aa, Homo sapiens
EVQLVESGGGLVQPGGSLRLSCAASGFSLSSHAMSWVRQAPGKGLEWIGTISTIDTTYYASWAKGRFTISRDNSKNTVYLQMNSLRAEDTAVYYCARLSELYTTNSYYSRWGQGTLVTVSSASTKGPSVFPLAPSSKSTSGGTAALGCLVKDYFPEPVTVSWNSGALTSGVHTFPAVLQSSGLYSLSSVVTVPSSSLGTQTYICNVNHKPSNTKVDKRVEPKSCDKTHTCPPCPAPEAAGGPSVFLFPPKPKDTLMISRTPEVTCVVVDVSHEDPEVKFNWYVDGVEVHNAKTKPREEQYASTYRVVSVLTVLHQDWLNGKEYKCKVSNKALPAPIEKTISKAKGQPREPQVYTLPPSREEMTKNQVSLTCLVKGFYPSDIAVEWESNGQPENNYKTTPPVLDSDGSFFLYSKLTVDKSRWQQGNVFSCSVMHEALHNHYTQKSLSLSPG

SEQ ID NO: 91 - protein, 480 aa, Homo sapiens
DIQMTQSPSSLSASVGDRVTITCQASESIGSLLAWYQQKPGKAPKLLIYRASTLESGVPSRFSGSGSGTDFTLTISSLQPEDFATYYCQSYHYSSSSSYAAFGQGTKVEIKRTVAAPSVFIFPPSDEQLKSGTASVVCLLNNFYPREAKVQWKVDNALQSGNSQESVTEQDSKDSTYSLSSTLTLSKADYEKHKVYACEVTHQGLSSPVTKSFNRGECGGGGSGGGGSDIQMTQSPSSLSASVGDRVTITCQSSESVYDNNYLSWYQQKPGKAPKLLIYDASRLASGVPSRFSGSGSGTDFTLTISSLQPEDFATYYCLGGYDSSGWYAAFGTGTKVTVLGGGGGSGGGGSGGGGSGGGGSEVQLVESGGGLVQPGGSLRLSCAASGFSLTIYTITWVRQAPGKGLEWIGTINSYGNTYYSTWAKGRFTISRDNSKNTVYLQMNSLRAEDTAVYYCARGYVDSDWYLNIWGQGTLVTVSS

SEQ ID NO: 92 - protein, 478 aa, Homo sapiens
DIQMTQSPSSLSASVGDRVTITCQASESIGSLLAWYQQKPGKAPKLLIYRASTLESGVPSRFSGSGSGTDFTLTISSLQPEDFATYYCQSYHYSSSSSYAAFGQGTKVEIKRTVAAPSVFIFPPSDEQLKSGTASVVCLLNNFYPREAKVQWKVDNALQSGNSQESVTEQDSKDSTYSLSSTLTLSKADYEKHKVYACEVTHQGLSSPVTKSFNRGECGGGGSGGGGSDIQMTQSPSSLSASVGDRVTITCQASQNIYRNLVWYQQKPGKAPKLLIYGASELESGVPSRFSGSGSGTDFTLTISSLQPEDFATYYCLSTYYISSSDNSFGTGTKVTVLGGGGGSGGGGSGGGGSGGGGSEVQLVESGGGLVQPGGSLRLSCAASGFSLSSYAMIWVRQAPGKGLEWIGFIDTDGHTEYANWAKGRFTISRDNSKNTVYLQMNSLRAEDTAVYYCARDGDHDYWGFNLWGQGTLVTVSS

SEQ ID NO: 93 - protein, 448 aa, Homo sapiens
EVQLVESGGGLVQPGGSLRLSCAASGFSLTIYTITWVRQAPGKGLEWIGTINSYGNTYYSTWAKGRFTISRDNSKNTVYLQMNSLRAEDTAVYYCARGYVDSDWYLNIWGQGTLVTVSSASTKGPSVFPLAPSSKSTSGGTAALGCLVKDYFPEPVTVSWNSGALTSGVHTFPAVLQSSGLYSLSSVVTVPSSSLGTQTYICNVNHKPSNTKVDKRVEPKSCDKTHTCPPCPAPEAAGGPSVFLFPPKPKDTLMISRTPEVTCVVVDVSHEDPEVKFNWYVDGVEVHNAKTKPREEQYASTYRVVSVLTVLHQDWLNGKEYKCKVSNKALPAPIEKTISKAKGQPREPQVYTLPPSREEMTKNQVSLTCLVKGFYPSDIAVEWESNGQPENNYKTTPPVLDSDGSFFLYSKLTVDKSRWQQGNVFSCSVMHEALHNHYTQKSLSLSPG

SEQ ID NO: 94 - protein, 479 aa, Homo sapiens
DIQMTQSPSSLSASVGDRVTITCQSSESVYDNNYLSWYQQKPGKAPKLLIYDASRLASGVPSRFSGSGSGTDFTLTISSLQPEDFATYYCLGGYDSSGWYAAFGQGTKVEIKRTVAAPSVFIFPPSDEQLKSGTASVVCLLNNFYPREAKVQWKVDNALQSGNSQESVTEQDSKDSTYSLSSTLTLSKADYEKHKVYACEVTHQGLSSPVTKSFNRGECGGGGSGGGGSDIQMTQSPSSLSASVGDRVTITCQASQSISSYLAWYQQKPGKAPKLLIYRASTLASGVPSRFSGSGSGTDFTLTISSLQPEDFATYYCQQAYSLSNVDNFFGTGTKVTVLGGGGGSGGGGSGGGGSGGGGSEVQLVESGGGLVQPGGSLRLSCAASGIDLSYYAMNWVRQAPGKGLEWIGMIVGGGITFYANWAKGRFTISRDNSKNTVYLQMNSLRAEDTAVYYCAVGSDGGISDFNIWGQGTLVTVSS

SEQ ID NO: 95 - protein, 482 aa, Homo sapiens
DIQMTQSPSSLSASVGDRVTITCQSSESVYDNNYLSWYQQKPGKAPKLLIYDASRLASGVPSRFSGSGSGTDFTLTISSLQPEDFATYYCLGGYDSSGWYAAFGQGTKVEIKRTVAAPSVFIFPPSDEQLKSGTASVVCLLNNFYPREAKVQWKVDNALQSGNSQESVTEQDSKDSTYSLSSTLTLSKADYEKHKVYACEVTHQGLSSPVTKSFNRGECGGGGSGGGGSDIQMTQSPSSLSASVGDRVTITCQASESIGSLLAWYQQKPGKAPKLLIYRASTLESGVPSRFSGSGSGTDFTLTISSLQPEDFATYYCQSYHYSSSSSYAAFGTGTKVTVLGGGGGSGGGGSGGGGSGGGGSEVQLVESGGGLVQPGGSLRLSCAASGFSLSSHAMSWVRQAPGKGLEWIGTISTIDTTYYASWAKGRFTISRDNSKNTVYLQMNSLRAEDTAVYYCARLSELYTTNSYYSRWGQGTLVTVSS

SEQ ID NO: 96 - protein, 448 aa, Homo sapiens
EVQLVESGGGLVQPGGSLRLSCAASGFSLSSYAMIWVRQAPGKGLEWIGFIDTDGHTEYANWAKGRFTISRDNSKNTVYLQMNSLRAEDTAVYYCARDGDHDYWGFNLWGQGTLVTVSSASTKGPSVFPLAPSSKSTSGGTAALGCLVKDYFPEPVTVSWNSGALTSGVHTFPAVLQSSGLYSLSSVVTVPSSSLGTQTYICNVNHKPSNTKVDKRVEPKSCDKTHTCPPCPAPEAAGGPSVFLFPPKPKDTLMISRTPEVTCVVVDVSHEDPEVKFNWYVDGVEVHNAKTKPREEQYASTYRVVSVLTVLHQDWLNGKEYKCKVSNKALPAPIEKTISKAKGQPREPQVYTLPPSREEMTKNQVSLTCLVKGFYPSDIAVEWESNGQPENNYKTTPPVLDSDGSFFLYSKLTVDKSRWQQGNVFSCSVMHEALHNHYTQKSLSLSPG

SEQ ID NO: 97 - protein, 480 aa, Homo sapiens
DIQMTQSPSSLSASVGDRVTITCQASQNIYRNLVWYQQKPGKAPKLLIYGASELESGVPSRFSGSGSGTDFTLTISSLQPEDFATYYCLSTYYISSSDNSFGQGTKVEIKRTVAAPSVFIFPPSDEQLKSGTASVVCLLNNFYPREAKVQWKVDNALQSGNSQESVTEQDSKDSTYSLSSTLTLSKADYEKHKVYACEVTHQGLSSPVTKSFNRGECGGGGSGGGGSDIQMTQSPSSLSASVGDRVTITCQASESIGSLLAWYQQKPGKAPKLLIYRASTLESGVPSRFSGSGSGTDFTLTISSLQPEDFATYYCQSYHYSSSSSYAAFGTGTKVTVLGGGGGSGGGGSGGGGSGGGGSEVQLVESGGGLVQPGGSLRLSCAASGFSLSSHAMSWVRQAPGKGLEWIGTISTIDTTYYASWAKGRFTISRDNSKNTVYLQMNSLRAEDTAVYYCARLSELYTTNSYYSRWGQGTLVTVSS

SEQ ID NO: 98 - protein, 712 aa, Homo sapiens
EVQLVESGGGLVQPGGSLRLSCAASGFSLSSHAMSWVRQAPGKGLEWIGTISTIDTTYYASWAKGRFTISRDNSKNTVYLQMNSLRAEDTAVYYCARLSELYTTNSYYSRWGQGTLVTVSSASTKGPSVFPLAPSSKSTSGGTAALGCLVKDYFPEPVTVSWNSGALTSGVHTFPAVLQSSGLYSLSSVVTVPSSSLGTQTYICNVNHKPSNTKVDKRVEPKSCDKTHTCPPCPAPEAAGGPSVFLFPPKPKDTLMISRTPEVTCVVVDVSHEDPEVKFNWYVDGVEVHNAKTKPREEQYASTYRVVSVLTVLHQDWLNGKEYKCKVSNKALPAPIEKTISKAKGQPREPQVYTLPPSREEMTKNQVSLTCLVKGFYPSDIAVEWESNGQPENNYKTTPPVLDSDGSFFLYSKLTVDKSRWQQGNVFSCSVMHEALHNHYTQKSLSLSPGGGGGSGGGGSAIQMTQSPSSLSARVGDRVTITCQSSESVYDNNYLSWYQQKPGKAPKLLIYDASRLASGVPSRFSGSGSGTQFTLTISSLQPEDFATYYCLGGYDSSGWYAAFGTGTKVTVLGGGGGSGGGGSGGGGSGGGGSEVQLVESGGGLVQPGGSLRLSCAASGFSLTIYTITWVRQAPGKGLEWIGTINSYGNTYYSTWAKGRFTISRDNSKNTVYLQMNSLRAEDTAVYYCARGYVDSDWYLNIWGQGTLVTVSS

SEQ ID NO: 99 - protein, 329 aa, Homo sapiens
ASTKGPSVFPLAPSSKSTSGGTAALGCLVKDYFPEPVTVSWNSGALTSGVHTFPAVLQSSGLYSLSSVVTVPSSSLGTQTYICNVNHKPSNTKVDKRVEPKSCDKTHTCPPCPAPEAAGGPSVFLFPPKPKDTLMISRTPEVTCVVVDVSHEDPEVKFNWYVDGVEVHNAKTKPREEQYNSTYRVVSVLTVLHQDWLNGKEYKCKVSNKALPAPIEKTISKAKGQPREPQVYTLPPSREEMTKNQVSLTCLVKGFYPSDIAVEWESNGQPENNYKTTPPVLDSDGSFFLYSKLTVDKSRWQQGNVFSCSVMHEALHNHYTQKSLSLSPG

SEQ ID NO: 100 - protein, 712 aa, Homo sapiens
EVQLVESGGGLVQPGGSLRLSCAASGFSLSSHAMSWVRQAPGKGLEWIGTISTIDTTYYASWAKGRFTISRDNSKNTVYLQMNSLRAEDTAVYYCARLSELYTTNSYYSRWGQGTLVTVSSASTKGPSVFPLAPSSKSTSGGTAALGCLVKDYFPEPVTVSWNSGALTSGVHTFPAVLQSSGLYSLSSVVTVPSSSLGTQTYICNVNHKPSNTKVDKRVEPKSCDKTHTCPPCPAPEAAGGPSVFLFPPKPKDTLMISRTPEVTCVVVDVSHEDPEVKFNWYVDGVEVHNAKTKPREEQYNSTYRVVSVLTVLHQDWLNGKEYKCKVSNKALPAPIEKTISKAKGQPREPQVYTLPPSREEMTKNQVSLTCLVKGFYPSDIAVEWESNGQPENNYKTTPPVLDSDGSFFLYSKLTVDKSRWQQGNVFSCSVMHEALHNHYTQKSLSLSPGGGGGSGGGGSDIQMTQSPSSLSASVGDRVTITCQSSESVYDNNYLSWYQQKPGKAPKLLIYDASRLASGVPSRFSGSGSGTDFTLTISSLQPEDFATYYCLGGYDSSGWYAAFGTGTKVTVLGGGGGSGGGGSGGGGSGGGGSEVQLVESGGGLVQPGGSLRLSCAASGFSLTIYTITWVRQAPGKGLEWIGTINSYGNTYYSTWAKGRFTISRDNSKNTVYLQMNSLRAEDTAVYYCARGYVDSDWYLNIWGQGTLVTVSS

SEQ ID NO: 101 - protein, 712 aa, Homo sapiens
EVQLVESGGGLVQPGGSLRLSCAASGFSLSSHAMSWVRQAPGKGLEWIGTISTIDTTYYASWAKGRFTISRDNSKNTVYLQMNSLRAEDTAVYYCARLSELYTTNSYYSRWGQGTLVTVSSASTKGPSVFPLAPSSKSTSGGTAALGCLVKDYFPEPVTVSWNSGALTSGVHTFPAVLQSSGLYSLSSVVTVPSSSLGTQTYICNVNHKPSNTKVDKRVEPKSCDKTHTCPPCPAPEAAGGPSVFLFPPKPKDTLMISRTPEVTCVVVDVSHEDPEVKFNWYVDGVEVHNAKTKPREEQYNSTYRVVSVLTVLHQDWLNGKEYKCKVSNKALPAPIEKTISKAKGQPREPQVYTLPPSREEMTKNQVSLTCLVKGFYPSDIAVEWESNGQPENNYKTTPPVLDSDGSFFLYSKLTVDKSRWQQGNVFSCSVMHEALHNHYTQKSLSLSPGGGGGSGGGGSAIQMTQSPSSLSARVGDRVTITCQSSESVYDNNYLSWYQQKPGKAPKLLIYDASRLASGVPSRFSGSGSGTQFTLTISSLQPEDFATYYCLGGYDSSGWYAAFGCGTKVTVLGGGGGSGGGGSGGGGSGGGGSEVQLVESGGGLVQPGGSLRLSCAASGFSLTIYTITWVRQAPGKCLEWIGTINSYGNTYYSTWAKGRFTISRDNSKNTVYLQMNSLRAEDTAVYYCARGYVDSDWYLNIWGQGTLVTVSS

SEQ ID NO: 102 - protein, 712 aa, Homo sapiens
EVQLVESGGGLVQPGGSLRLSCAASGFSLSSHAMSWVRQAPGKGLEWIGTISTIDTTYYASWAKGRFTISRDNSKNTVYLQMNSLRAEDTAVYYCARLSELYTTNSYYSRWGQGTLVTVSSASTKGPSVFPLAPSSKSTSGGTAALGCLVKDYFPEPVTVSWNSGALTSGVHTFPAVLQSSGLYSLSSVVTVPSSSLGTQTYICNVNHKPSNTKVDKRVEPKSCDKTHTCPPCPAPEAAGGPSVFLFPPKPKDTLMISRTPEVTCVVVDVSHEDPEVKFNWYVDGVEVHNAKTKPREEQYNSTYRVVSVLTVLHQDWLNGKEYKCKVSNKALPAPIEKTISKAKGQPREPQVYTLPPSREEMTKNQVSLTCLVKGFYPSDIAVEWESNGQPENNYKTTPPVLDSDGSFFLYSKLTVDKSRWQQGNVFSCSVMHEALHNHYTQKSLSLSPGGGGGSGGGGSAIQMTQSPSSLSARVGDRVTITCQSSESVYDNNYLSWYQQKPGKAPKLLIYDASRLASGVPSRFSGSGSGTQFTLTISSLQPEDFATYYCLGGYDSSGWYAAFGTGTKVTVLGGGGGSGGGGSGGGGSGGGGSEVQLVESGGGLVQPGGSLRLSCAASGFSLTIYTITWVRQAPGKGLEWIGTINSYGNTYYSTWAKGRFTISRDNSKNTVYLQMNSLRAEDTAVYYCARGYVDSDWYLNIWGQGTLVTVSS

SEQ ID NO: 103 - protein, 711 aa, Homo sapiens
EVQLVESGGGLVQPGGSLRLSCAASGFSLTIYTITWVRQAPGKGLEWIGTINSYGNTYYSTWAKGRFTISRDNSKNTVYLQMNSLRAEDTAVYYCARGYVDSDWYLNIWGQGTLVTVSSASTKGPSVFPLAPSSKSTSGGTAALGCLVKDYFPEPVTVSWNSGALTSGVHTFPAVLQSSGLYSLSSVVTVPSSSLGTQTYICNVNHKPSNTKVDKRVEPKSCDKTHTCPPCPAPEAAGGPSVFLFPPKPKDTLMISRTPEVTCVVVDVSHEDPEVKFNWYVDGVEVHNAKTKPREEQYNSTYRVVSVLTVLHQDWLNGKEYKCKVSNKALPAPIEKTISKAKGQPREPQVYTLPPSREEMTKNQVSLTCLVKGFYPSDIAVEWESNGQPENNYKTTPPVLDSDGSFFLYSKLTVDKSRWQQGNVFSCSVMHEALHNHYTQKSLSLSPGGGGGSGGGGSDIQMTQSPSSLSASVGDRVTITCQASESIGSLLAWYQQKPGKAPKLLIYRASTLESGVPSRFSGSGSGTDFTLTISSLQPEDFATYYCQSYHYSSSSSYAAFGCGTKVTVLGGGGGSGGGGSGGGGSGGGGSEVQLVESGGGLVQPGGSLRLSCAASGFSLSSHAMSWVRQAPGKCLEWIGTISTIDTTYYASWAKGRFTISRDNSKNTVYLQMNSLRAEDTAVYYCARLSELYTTNSYYSRWGQGTLVTVSS

SEQ ID NO: 104 - protein, 112 aa, Homo sapiens
DIQMTQSPSSLSASVGDRVTITCQSSQSVDNNNWLAWYQQKPGKAPKLLIYDASTLASGVPSRFSGSGSGTDFTLTISSLQPEDFATYYCQGTYYTTDWWNSFGQGTKVEIK

SEQ ID NO: 105 - protein, 111 aa, Homo sapiens
DIQMTQSPSSLSASVGDRVTITCQASQDIESYLNWYQQKPGKAPKLLIYYASTLASGVPSRFSGSGSGTDFTLTISSLQPEDFATYYCQQSYSNSDVDKNVFGQGTKVEIK

SEQ ID NO: 106 - protein, 112 aa, Homo sapiens
DIQMTQSPSSLSASVGDRVTITCQSSESVYDNNYLSWYQQKPGKAPKLLIYDASRLASGVPSRFSGSGSGTDFTLTISSLQPEDFATYYCLGGYDSSGWYAAFGQGTKVEIK

SEQ ID NO: 107 - protein, 112 aa, Homo sapiens
AIQMTQSPSSLSARVGDRVTITCQSSESVYDNNYLSWYQQKPGKAPKLLIYDASRLASGVPSRFSGSGSGTQFTLTISSLQPEDFATYYCLGGYDSSGWYAAFGQGTKVEIK

SEQ ID NO: 108 - protein, 112 aa, Homo sapiens; identical to SEQ ID NO: 107

SEQ ID NO: 109 - protein, 110 aa, Homo sapiens
DIQMTQSPSSLSASVGDRVTITCQASQNIYRNLVWYQQKPGKAPKLLIYGASELESGVPSRFSGSGSGTDFTLTISSLQPEDFATYYCLSTYYISSSDNSFGQGTKVEIK

SEQ ID NO: 110 - protein, 111 aa, Homo sapiens
DIQMTQSPSSLSASVGDRVTITCQASQSIGAYLSWYQQKPGKAPKLLIYEASTLASGVPSRFSGSGSGTDFTLTISSLQPEDFATYYCLGAYGRSSDDGTAFGQGTKVEIK

SEQ ID NO: 111 - protein, 110 aa, Homo sapiens
DVQMTQSPSSLSASVGDRVTITCQASQNTYSNLDWYQQKPGKAPKLLIYQASKLASGVPSRFSGSGSGTDFTLTISSLQPEDFATYYCQSTSWGSSYVGGFGQGTKVEIK

SEQ ID NO: 112 - protein, 110 aa, Homo sapiens
DIQMTQSPSSLSASVGDRVTITCQASQSISSYLAWYQQKPGKAPKLLIYRASTLASGVPSRFSGSGSGTDFTLTISSLQPEDFATYYCQQAYSLSNVDNFFGQGTKVEIK

SEQ ID NO: 113 - protein, 111 aa, Homo sapiens
DIQMTQSPSSLSASVGDRVTITCQASESIGSLLAWYQQKPGKAPKLLIYRASTLESGVPSRFSGSGSGTDFTLTISSLQPEDFATYYCQSYHYSSSSSYAAFGQGTKVEIK

SEQ ID NO: 114 - protein, 111 aa, Homo sapiens; identical to SEQ ID NO: 113

SEQ ID NO: 115 - protein, 343 aa, Homo sapiens
MWSHLNRLLFWSIFSSVTCRKAVLDCEAMKTNEFPSPCLDSKTKVVMKGQNVSMFCSHKNKSLQITYSLFRRKTHLGTQDGKGEPAIFNLSITEAHESGPYKCKAQVTSCSKYSRDFSFTIVDPVTSPVLNIMVIQTETDRHITLHCLSVNGSLPINYTFFENHVAISPAISKYDREPAEFNLTKKNPGEEEEYRCEAKNRLPNYATYSHPVTMPSTGGDSCPFCLKLLLPGLLLLLVVIILILAFWVLPKYKTRKAMRNNVPRDRGDTAMEVGIYANILEKQAKEESVPEVGSRPCVSTAQDEAKHSQELQYATPVFQEVAPREQEACDSYKSGYVYSELNF